European Patent Application EP 4 193 830 A2, published June 14, 2023. Title: Lettuce Plants Having Resistance to Downy Mildew. Applicant: Seminis Vegetable Seeds, Inc. The sequence listing filed with the application follows.

SEQUENCE LISTING (85 sequences)

SEQ ID NO: 1 - DNA, 228 bp, Lactuca sativa
  source 1..228: mol_type = genomic DNA
gattccgatgttctaattttactcaacagatatcccccgccttaacataggtacacatttgaaacacccctttnatntctctcctaatagctcctytgcaacatcctccattaatcttccgnctccttgtcttttctagnagcacgtgttgtcgtggntaacaagnacccctaaccttcatcggacatcttcaacaacngncgacgacttcacagttttgaggtttct

SEQ ID NO: 2 - DNA, 25 bp, synthetic construct
  source 1..25: mol_type = other DNA; note = Primer
aggtacacatttgaaacaccccttt

SEQ ID NO: 3 - DNA, 25 bp, synthetic construct
  source 1..25: mol_type = other DNA; note = Primer
ttgaagatgtccgatgaaggttagg

SEQ ID NO: 4 - DNA, 16 bp, synthetic construct
  source 1..16: mol_type = other DNA; note = Probe
atgttgcagaggagct

SEQ ID NO: 5 - DNA, 16 bp, synthetic construct
  source 1..16: mol_type = other DNA; note = Probe
atgttgcaaaggagct

SEQ ID NO: 6 - DNA, 87 bp, Lactuca sativa
  source 1..87: mol_type = genomic DNA
acttttgagctttcaacacatccaagtagtgaaatgttactaawtacntgtaggttgggccagaatatgcaagatattgtgggatag

SEQ ID NO: 7 - DNA, 25 bp, synthetic construct
  source 1..25: mol_type = other DNA; note = Primer
acttttgagctttcaacacatccaa

SEQ ID NO: 8 - DNA, 22 bp, synthetic construct
  source 1..22: mol_type = other DNA; note = Primer
gcatattctggcccaacctaca

SEQ ID NO: 9 - DNA, 20 bp, synthetic construct
  source 1..20: mol_type = other DNA; note = Probe
agtgaaatgttactaaatac

SEQ ID NO: 10 - DNA, 20 bp, synthetic construct
  source 1..20: mol_type = other DNA; note = Probe
agtgaaatgttactaattac

SEQ ID NO: 11 - DNA, 111 bp, Lactuca sativa
  source 1..111: mol_type = genomic DNA
ttgacctgatttgacctcctttacttaaccttgaccngttgactttccctttctttgyatatctaatcnttatatgatgtacaccaaaatattaacctatttcacttcatt

SEQ ID NO: 12 - DNA, 25 bp, synthetic construct
  source 1..25: mol_type = other DNA; note = Primer
ttgacctgatttgacctcctttact

SEQ ID NO: 13 - DNA, 34 bp, synthetic construct
  source 1..34: mol_type = other DNA; note = Primer
aatgaagtgaaataggttaatattttggtgtaca

SEQ ID NO: 14 - DNA, 18 bp, synthetic construct
  source 1..18: mol_type = other DNA; note = Probe
ccctttctttgcatatct

SEQ ID NO: 15 - DNA, 19 bp, synthetic construct
  source 1..19: mol_type = other DNA; note = Probe
tccctttctttgtatatct

SEQ ID NO: 16 - DNA, 204 bp, Lactuca sativa
  source 1..204: mol_type = genomic DNA
cttaaagatgctgtaaaagagcttttagggccggagatatcaagcaatgtagttatygagcattcgaaaganggatctggtattggagctgcactcttagcngctacaaactcgatttacgaacattaattgtatattgtgagggtaattattggcccaaaactaaatatgtattgaatgtatcttatgtgtaatttttataaa

SEQ ID NO: 17 - DNA, 21 bp, synthetic construct
  source 1..21: mol_type = other DNA; note = Primer
gggccggagatatcaagcaat

SEQ ID NO: 18 - DNA, 22 bp, synthetic construct
  source 1..22: mol_type = other DNA; note = Primer
agtgcagctccaataccagatc

SEQ ID NO: 19 - DNA, 17 bp, synthetic construct
  source 1..17: mol_type = other DNA; note = Probe
cgaatgctcgataacta

SEQ ID NO: 20 - DNA, 18 bp, synthetic construct
  source 1..18: mol_type = other DNA; note = Probe
tcgaatgctcaataacta

SEQ ID NO: 21 - DNA, 201 bp, Lactuca sativa
  source 1..201: mol_type = genomic DNA
tttaggaagacgcaagaatgaatttatggcgatggacaagacaactaaggcgaattaataaatgaaaggtcgacaaaaacaaagaaagacaaagggttgawtgacatgtacaatttattaatattaaaataaatggacagacggcaaattttcatttcaagttttatttaaatatttttatatcagtccctgcgatttgca

SEQ ID NO: 22 - DNA, 30 bp, synthetic construct
  source 1..30: mol_type = other DNA; note = Primer
ggcgaattaataaatgaaaggtcgacaaaa

SEQ ID NO: 23 - DNA, 29 bp, synthetic construct
  source 1..29: mol_type = other DNA; note = Primer
atgaaaatttgccgtctgtccatttattt

SEQ ID NO: 24 - DNA, 19 bp, synthetic construct
  source 1..19: mol_type = other DNA; note = Probe
acaaagggttgaatgacat

SEQ ID NO: 25 - DNA, 19 bp, synthetic construct
  source 1..19: mol_type = other DNA; note = Probe
acaaagggttgattgacat

SEQ ID NO: 26 - DNA, 201 bp, Lactuca sativa
  source 1..201: mol_type = genomic DNA
ctataaaattatgaaaatacacatatttttccttgacaaaacattatgacaaagtaaacatcataatgcatggatcatgtaaactcacctgacccgttgcracaatgacaggatccctcatcatttccaaagtgattggacacaaaaactcaaatggaatcgtgatagacgcacatttttgtagcgttctattacatggag

SEQ ID NO: 27 - DNA, 30 bp, synthetic construct
  source 1..30: mol_type = other DNA; note = Primer
gacaaagtaaacatcataatgcatggatca

SEQ ID NO: 28 - DNA, 25 bp, synthetic construct
  source 1..25: mol_type = other DNA; note = Primer
cactttggaaatgatgagggatcct

SEQ ID NO: 29 - DNA, 14 bp, synthetic construct
  source 1..14: mol_type = other DNA; note = Probe
ccgttgcaacaatg

SEQ ID NO: 30 - DNA, 14 bp, synthetic construct
  source 1..14: mol_type = other DNA; note = Probe
ccgttgcgacaatg

SEQ ID NO: 31 - DNA, 201 bp, Lactuca sativa
  source 1..201: mol_type = genomic DNA
gtttttaattaatttgattgatttattaaaacagatttatttaatatttgagaaaaaaacagaacattttcgtgttttttgaagcgtgatcatttattaaytttcatctctgttttcagaagaaccgtatttctactatttttagagaattcaattcaatttgaaggaaaaagcacaaatacgaataattgaaagacatta

SEQ ID NO: 32 - DNA, 25 bp, synthetic construct
  source 1..25: mol_type = other DNA; note = Primer
tttcgtgttttttgaagcgtgatca

SEQ ID NO: 33 - DNA, 37 bp, synthetic construct
  source 1..37: mol_type = other DNA; note = Primer
tgaattctctaaaaatagtagaaatacggttcttctg

SEQ ID NO: 34 - DNA, 21 bp, synthetic construct
  source 1..21: mol_type = other DNA; note = Probe
aaacagagatgaaagttaata

SEQ ID NO: 35 - DNA, 19 bp, synthetic construct
  source 1..19: mol_type = other DNA; note = Probe
acagagatgaaaattaata

SEQ ID NO: 36 - DNA, 121 bp, Lactuca sativa
  source 1..121: mol_type = genomic DNA
aatgcatcggacacacacctcgtgcgcaaacaggtctttcactgcgtgagcaggtagttcytgcacggcatatccaagaagcttcatctcgtccgcggccgctattgcgggatcttgatcg

SEQ ID NO: 37 - DNA, 20 bp, synthetic construct
  source 1..20: mol_type = other DNA; note = Primer
gcgcaaacaggtctttcact

SEQ ID NO: 38 - DNA, 25 bp, synthetic construct
  source 1..25: mol_type = other DNA; note = Primer
ggacgagatgaagcttcttggatat

SEQ ID NO: 39 - DNA, 14 bp, synthetic construct
  source 1..14: mol_type = other DNA; note = Probe
ccgtgcaagaacta

SEQ ID NO: 40 - DNA, 14 bp, synthetic construct
  source 1..14: mol_type = other DNA; note = Probe
ccgtgcaggaacta

SEQ ID NO: 41 - DNA, 280 bp, Lactuca sativa
  source 1..280: mol_type = genomic DNA
gttgtggaggcctatgtagatggcagatgtttggtcttgtggggttacattgtatgtgatgcttgttggtgcttatccwttcgaagatgaagatgatccnaaaaanttccgaaaaacactcacngtgagtcttttanaaagnttnttattnttattnttatttctaaaagaaaanttnagtntcttcaactttnttcttgtttatcnttataaattaagaacattgtattaacatactatggcagcgtatacttagtgtccaatattcaatcccagacta

SEQ ID NO: 42 - DNA, 24 bp, synthetic construct
  source 1..24: mol_type = other DNA; note = Primer
gggttacattgtatgtgatgcttg

SEQ ID NO: 43 - DNA, 29 bp, synthetic construct
  source 1..29: mol_type = other DNA; note = Primer
cgctgccatagtatgttaatacaatgttc

SEQ ID NO: 44 - DNA, 20 bp, synthetic construct
  source 1..20: mol_type = other DNA; note = Probe
ttggtgcttatccattcgaa

SEQ ID NO: 45 - DNA, 20 bp, synthetic construct
  source 1..20: mol_type = other DNA; note = Probe
ttggtgcttatcctttcgaa

SEQ ID NO: 46 - DNA, 201 bp, Lactuca sativa
  source 1..201: mol_type = genomic DNA
ggaaaatatgtaaacgtgatgcttaataatttcatgatcttttgatgaatgcacacagattaactccagggagaaggtgaaggagttagataagaaagcawtgcaattgaattttgattacgaaaatggtggtttgagtatcttgcaattacttgaacaaatagatgatatcgaaaggttgggccttgactatcggtttca

SEQ ID NO: 47 - DNA, 24 bp, synthetic construct
  source 1..24: mol_type = other DNA; note = Primer
agggagaaggtgaaggagttagat

SEQ ID NO: 48 - DNA, 26 bp, synthetic construct
  source 1..26: mol_type = other DNA; note = Primer
caagatactcaaaccaccattttcgt

SEQ ID NO: 49 - DNA, 17 bp, synthetic construct
  source 1..17: mol_type = other DNA; note = Probe
tcaattgcattgctttc

SEQ ID NO: 50 - DNA, 16 bp, synthetic construct
  source 1..16: mol_type = other DNA; note = Probe
caattgcaatgctttc

SEQ ID NO: 51 - DNA, 194 bp, Lactuca sativa
  source 1..194: mol_type = genomic DNA
gacggtttcatctccgtggagtacgattgtgcagggntcgccggtcatggtaccggatgctgtttccgnggcgccggtttctgttgytccagcaccgacgttttcatcttctgttgaggagaaaataggtaactttacctcggattggtgtccgccttcaatggtgccggatgtagtaagctctccggatgatt

SEQ ID NO: 52 - DNA, 20 bp, synthetic construct
  source 1..20: mol_type = other DNA; note = Primer
tggtaccggatgctgtttcc

SEQ ID NO: 53 - DNA, 26 bp, synthetic construct
  source 1..26: mol_type = other DNA; note = Primer
ttctcctcaacagaagatgaaaacgt

SEQ ID NO: 54 - DNA, 15 bp, synthetic construct
  source 1..15: mol_type = other DNA; note = Probe
tgctggagcaacaga

SEQ ID NO: 55 - DNA, 15 bp, synthetic construct
  source 1..15: mol_type = other DNA; note = Probe
tgctggaacaacaga

SEQ ID NO: 56 - DNA, 201 bp, Lactuca sativa
  source 1..201: mol_type = genomic DNA
atgttatacattggtctcacacctagttaaagaatatgttgttgtgaacatacctaaaaccaaacacaaatttgctaccattttatagatgacattaaacratttattatgtgttgtctagagataacgagaataagcattttagtggaataaatcattatgtcccatcatcaaatcatgtttggttagtctttgcacact

SEQ ID NO: 57 - DNA, 28 bp, synthetic construct
  source 1..28: mol_type = other DNA; note = Primer
gttgtgaacatacctaaaaccaaacaca

SEQ ID NO: 58 - DNA, 29 bp, synthetic construct
  source 1..29: mol_type = other DNA; note = Primer
gcttattctcgttatctctagacaacaca

SEQ ID NO: 59 - DNA, 20 bp, synthetic construct
  source 1..20: mol_type = other DNA; note = Probe
atgacattaaacgatttatt

SEQ ID NO: 60 - DNA, 20 bp, synthetic construct
  source 1..20: mol_type = other DNA; note = Probe
atgacattaaacaatttatt

SEQ ID NO: 61 - DNA, 618 bp, Lactuca sativa
  source 1..618: mol_type = genomic DNA
gtgttccaaatctccgacatcatggtggcgttgtccgtcgatcggccatgagtttcccgagtcttcaacgaatcacaaccgctcttaatcgatctcatcgcaatccaattcaattttcagtcagaagcacaagttatctagatctaagtcttgattttaatttcaacatcaccatggatgattctcatactaagaaggaagtccaatctggtgatggcttgaacgttgttaaggatacaaaggaaacgaaaaagtcgccggagatccctccgccaccgaagaaaccattgccgggagattgctgtggcagtggttgtgttcgctgcgtntgggacntatattatgatgagcttgnagaatataacaaacttctaaagggagnatccgattcttcantcggatcnaaggtttcttaacattatgcacaaattaatcgatttttgtcncatatagatctgtttgattttcatgtatacaattcaattggatatgtttaytgnaatcttatgaacttcactaggtgctatataactcgatgcatctgaaaataccaatcggttngagatgattattgnancccattgaataattcgatttaaattcatgatcttgactcat

SEQ ID NO: 62 - DNA, 32 bp, synthetic construct
  source 1..32: mol_type = other DNA; note = Primer
aaggtttcttaacattatgcacaaattaatcg

SEQ ID NO: 63 - DNA, 27 bp, synthetic construct
  source 1..27: mol_type = other DNA; note = Primer
tgcatcgagttatatagcacctagtga

SEQ ID NO: 64 - DNA, 21 bp, synthetic construct
  source 1..21: mol_type = other DNA; note = Probe
ttcaattggatatgtttactg

SEQ ID NO: 65 - DNA, 19 bp, synthetic construct
  source 1..19: mol_type = other DNA; note = Probe
caattggatatgtttattg

SEQ ID NO: 66 - DNA, 121 bp, Lactuca sativa
  source 1..121: mol_type = genomic DNA
catccatcgntggtgaatgaaatctctgttgtccttgattaccatgttcaaaggagcttcyactgaaattagacatgccaaattgctgacttgcaggaaatccaggattttgatgactcgt

SEQ ID NO: 67 - DNA, 27 bp, synthetic construct
  source 1..27: mol_type = other DNA; note = Primer
ctctgttgtccttgattaccatgttca

SEQ ID NO: 68 - DNA, 22 bp, synthetic construct
  source 1..22: mol_type = other DNA; note = Primer
gcaagtcagcaatttggcatgt

SEQ ID NO: 69 - DNA, 19 bp, synthetic construct
  source 1..19: mol_type = other DNA; note = Probe
ctaatttcagtagaagctc

SEQ ID NO: 70 - DNA, 14 bp, synthetic construct
  source 1..14: mol_type = other DNA; note = Probe
ttcagtggaagctc

SEQ ID NO: 71 - DNA, 201 bp, Lactuca sativa
  source 1..201: mol_type = genomic DNA
tctcaattcgtttcgagatggaattacagatctttatgctgaccaacattctggagtacaaatcgttgacttggtcttcnattccatgcttgttgctaccrttttcaccgcttaattgggaagattttcgatcgtaaagcttcttaatttcactaccagcctataaaatgtcgaaatcattgataataactcaacaaatgc

SEQ ID NO: 72 - DNA, 25 bp, synthetic construct
  source 1..25: mol_type = other DNA; note = Primer
accaacattctggagtacaaatcgt

SEQ ID NO: 73 - DNA, 29 bp, synthetic construct
  source 1..29: mol_type = other DNA; note = Primer
atttcgacattttataggctggtagtgaa

SEQ ID NO: 74 - DNA, 16 bp, synthetic construct
  source 1..16: mol_type = other DNA; note = Probe
ttgctaccattttcac

SEQ ID NO: 75 - DNA, 15 bp, synthetic construct
  source 1..15: mol_type = other DNA; note = Probe
tgctaccgttttcac

SEQ ID NO: 76 - DNA, 201 bp, Lactuca sativa
  source 1..201: mol_type = genomic DNA
accctctgtacattcttccactccatatatctctccacaaatgtctgttccagttcgcccttttggcaacaacatgatgtatcatggtaggaatatcttcyacagttatttatcattctactttgtgttatttcaaatttgtgaatctttttttgcagatatgtctcctgtgttctatgtacaaggtccaccacctccacc

SEQ ID NO: 77 - DNA, 25 bp, synthetic construct
  source 1..25: mol_type = other DNA; note = Primer
cccttttggcaacaacatgatgtat

SEQ ID NO: 78 - DNA, 31 bp, synthetic construct
  source 1..31: mol_type = other DNA; note = Primer
ggagacatatctgcaaaaaaagattcacaaa

SEQ ID NO: 79 - DNA, 23 bp, synthetic construct
  source 1..23: mol_type = other DNA; note = Probe
aatgataaataactgtagaagat

SEQ ID NO: 80 - DNA, 21 bp, synthetic construct
  source 1..21: mol_type = other DNA; note = Probe
tgataaataactgtggaagat

SEQ ID NO: 81 - DNA, 201 bp, Lactuca sativa
  source 1..201: mol_type = genomic DNA
cagatttccttctgtattcttaaaagggattaaacgtacgtcgaggtaaaactactaaattttatgtcatacatgaattcattcctatattcaggagtgcycgtttgaaaagggttgtcttatatacatgaatcaattcgtgtattacactcaaatcagtaaataaacgattattaaaaaaaatatttgatatcgtaacaa

SEQ ID NO: 82 - DNA, 43 bp, synthetic construct
  source 1..43: mol_type = other DNA; note = Primer
actactaaattttatgtcatacatgaattcattcctatattca

SEQ ID NO: 83 - DNA, 28 bp, synthetic construct
  source 1..28: mol_type = other DNA; note = Primer
acaaatacgatgggattgattgttacga

SEQ ID NO: 84 - DNA, 16 bp, synthetic construct
  source 1..16: mol_type = other DNA; note = Probe
ttcaaacgggcactcc

SEQ ID NO: 85 - DNA, 16 bp, synthetic construct
  source 1..16: mol_type = other DNA; note = Probe
ttcaaacgagcactcc